European Patent Specification EP 3 658 913 B1, published April 3, 2024. Title: Méthode pour mesurer la modulation de l'activation d'un récepteur couplé à une protéine G. Applicant: CISBIO BIOASSAY CISBIO BIOASSAYS. The sequence listing filed with the application follows.

SEQUENCE LISTING (9 sequences)

SEQ ID NO: 1 - protein, 19 aa, Artificial Sequence
  Peptide KB1753
SSRGYYHGIWVGEEGRLSR

SEQ ID NO: 2 - protein, 143 aa, Artificial Sequence
  F11
EVQLVESGGGLVQPGGSLRLSCEASGFAFSDTWMYWVRQAPGKGLEWVATITRGDQNTYYTESVKGRFTISRDNAKNTLYLQMNSLKSEDTAVYYCAKEGPIGPPDYWGQGTQVTVSSAAAEQKLISEEDLNGAAHHHHHHGS

SEQ ID NO: 3 - protein, 143 aa, Artificial Sequence
  F4
EVQLVESGGGLVQPGGSLRLSCAASGFTFSSYYMNWVRQAPGKGLEWVSSIYNGDGDTDYSDSVKGRFTISRDNAKNTVYLEMSDLKVQDTAIYYCNAYDGTLLRDYWGQGTQVTVSSAAAEQKLISEEDLNGAAHHHHHHGS

SEQ ID NO: 4 - protein, 145 aa, Artificial Sequence
  G6
EVQLVESGGDLVQPGGSLRLSCAASGFTFSTYRMNWVRQAPGKGLEWVASISSRGITTDYAHPVKGRFTVSRDNTKNTLYLQMNSLKPDDAAVYYCATDPSTWYRGTAHWGQGTQVTVSSAAAEQKLISEEDLNGAAHHHHHHGS

SEQ ID NO: 5 - protein, 143 aa, Artificial Sequence
  B11
EVQLVESGGGLVQPGGSLRLSCAASGFTFNDYWMYWVRQAPGKGLEWVSSINTGGSSTYYSDSVKGRFTTARDNAKNSLYLQLNSLRPEDTAVYYCAKEGPVGPPDYWGQGTQVTVSSAAAEQKLISEEDLNGAAHHHHHHGS

SEQ ID NO: 6 - protein, 145 aa, Artificial Sequence
  F9
EVQLVESGGGLVQPGGSLRLSCAASGFTFDDYAMNWVRQAAGKGPEWVASISSRGITTDYAHSVKGRFTVSRDNTKNTLYLQMNSLKPDDAAVYYCATDPSTWYRGTAHWGQGTQVTVSSAAAEQKLISEEDLNGAAHHHHHHGS

SEQ ID NO: 7 - protein, 148 aa, Artificial Sequence
  G7
QVQLQESGGGLVQPGGSLRLSCAASGFTFSWYGMSWVRQAPGKGPEWVASISSRGITTDYAHSVKGRFTVSRDNTKNTLYLQMNSLKPEDTGVYYCTRVLWYDSGAYSLNDFWGQGTQVTVSSAAAEQKLISEEDLNGAAHHHHHHGS

SEQ ID NO: 8 - protein, 142 aa, Artificial Sequence
  A10
EVQLVESGGGLVQPGGSLRLSCAASGLTYSDYAMSWVRQAAGKGPEWVASISSRGITTDYAHSVKGRFTVSRDNTKNTLYLQMNSLEPEDTAVYYCTTVSYWRYEYWGQGTQVTVSSAAAEQKLISEEDLNGAAHHHHHHGS

SEQ ID NO: 9 - protein, 148 aa, Artificial Sequence
  E2
EVQLVESGGGLVQPGGSLRLSCIGSGYTFSSYAMAWVRQASGKGPEWVASISSRGITTDYAHSVKGRFTISRDNAKNTLYLHMNNLKPEDTALYYCTRVLWYENGLYSLNDFWGQGTQVTVSSAAAEQKLISEEDLNGAAHHHHHHGS